European Patent Application EP 4 711 455 A1, published March 18, 2026. Title: SMALL ARTIFICIAL RNA (smartRNA) OLIGONUCLEOTIDE FOR MODULATING PROTEIN EXPRESSION. Applicant: Aarhus Universitet. The sequence listing filed with the application follows.

SEQUENCE LISTING (192 sequences)

SEQ ID NO: 1 - protein, 321 aa, Homo sapiens
MKPGFSPRGGGFGGRGGFGDRGGRGGRGGFGGGRGRGGGFRGRGRGGGGGGGGGGGGGRGGGGFHSGGNRGRGRGGKRGNQSGKNVMVEPHRHEGVFICRGKEDALVTKNLVPGESVYGEKRVSISEGDDKIEYRAWNPFRSKLAAAILGGVDQIHIKPGAKVLYLGAASGTTVSHVSDIVGPDGLVYAVEFSHRSGRDLINLAKKRTNIIPVIEDARHPHKYRMLIAMVDVIFADVAQPDQTRIVALNAHTFLRNGGHFVISIKANCIDSTASAEAVFASEVKKMQQENMKPQEQLTLEPYERDHAVVVGVYRPPPKVKN

SEQ ID NO: 2 - protein, 594 aa, Homo sapiens
MVLLHVLFEHAVGYALLALKEVEEISLLQPQVEESVLNLGKFHSIVRLVAFCPFASSQVALENANAVSEGVVHEDLRLLLETHLPSKKKKVLLGVGDPKIGAAIQEELGYNCQTGGVIAEILRGVRLHFHNLVKGLTDLSACKAQLGLGHSYSRAKVKFNVNRVDNMIIQSISLLDQLDKDINTFSMRVREWYGYHFPELVKIINDNATYCRLAQFIGNRRELNEDKLEKLEELTMDGAKAKAILDASRSSMGMDISAIDLINIESFSSRVVSLSEYRQSLHTYLRSKMSQVAPSLSALIGEAVGARLIAHAGSLTNLAKYPASTVQILGAEKALFRALKTRGNTPKYGLIFHSTFIGRAAAKNKGRISRYLANKCSIASRIDCFSEVPTSVFGEKLREQVEERLSFYETGEIPRKNLDVMKEAMVQAEEAAAEITRKLEKQEKKRLKKEKKRLAALALASSENSSSTPEECEEMSEKPKKKKKQKPQEVPQENGMEDPSISFSKPKKKKSFSKEELMSSDLEETAGSTSIPKRKKSTPKEETVNDPEEAGHRSGSKKKRKFSKEEPVSSGPEEAVGKSSSKKKKKFHKASQED

SEQ ID NO: 3 - protein, 529 aa, Homo sapiens
MLVLFETSVGYAIFKVLNEKKLQEVDSLWKEFETPEKANKIVKLKHFEKFQDTAEALAAFTALMEGKINKQLKKVLKKIVKEAHEPLAVADAKLGGVIKEKLNLSCIHSPVVNELMRGIRSQMDGLIPGVEPREMAAMCLGLAHSLSRYRLKFSADKVDTMIVQAISLLDDLDKELNNYIMRCREWYGWHFPELGKIISDNLTYCKCLQKVGDRKNYASAKLSELLPEEVEAEVKAAAEISMGTEVSEEDICNILHLCTQVIEISEYRTQLYEYLQNRMMAIAPNVTVMVGELVGARLIAHAGSLLNLAKHAASTVQILGAEKALFRALKSRRDTPKYGLIYHASLVGQTSPKHKGKISRMLAAKTVLAIRYDAFGEDSSSAMGVENRAKLEARLRTLEDRGIRKISGTGKALAKTEKYEHKSEVKTYDPSGDSTLPTCSKKRKIEQVDKEDEITEKKAKKAKIKVKVEEEEEEKVAEEEETSVKKKKKRGKKKHIKEEPLSEEEPCTSTAIASPEKKKKKKKKRENED

SEQ ID NO: 4 - protein, 128 aa, Homo sapiens
MTEADVNPKAYPLADAHLTKKLLDLVQQSCNYKQLRKGANEATKTLNRGISEFIVMAADAEPLEIILHLPLLCEDKNVPYVFVRSKQALGRACGVSRPVIACSVTIKEGSQLKQQIQSIQQSIERLLV

SEQ ID NO: 5 - RNA, 126 nt, Homo sapiens
  source 1..126: mol_type = other RNA
tcccaatgaagaaactttcacatgtcttactctctgtcctagtcccagagcctgtaaaggtgaacccactgggactggctgggggagaagaggaagatttgttccagaaggaactgtctgagggat

SEQ ID NO: 6 - RNA, 80 nt, synthetic construct
  source 1..80: mol_type = other RNA
ggatcacggtgatgagagctcggtacctctgacctcaggcctctgaggggtgatgaacttgttgatggtctgagtgatca

SEQ ID NO: 7 - RNA, 78 nt, synthetic construct
  source 1..78: mol_type = other RNA
gatcacggtgatgagatttttttttttctgacctcaggcctctgaggggtgatgaacttgttgatggtctgagtgatc

SEQ ID NO: 8 - RNA, 78 nt, synthetic construct
  source 1..78: mol_type = other RNA
gatcacggtgatgagagctcggtacctctgacctcaggcctctgaggggtgatgaactttttttttttctgagtgatc

SEQ ID NO: 9 - RNA, 88 nt, synthetic construct
  source 1..88: mol_type = other RNA
gatcacggtgatgagatttttttttttctgacctcaggcctctgaggggtgatgaactcgaggcggattcacccttgtctgagtgatc

SEQ ID NO: 10 - RNA, 88 nt, synthetic construct
  source 1..88: mol_type = other RNA
gatcacggtgatgagatcgaggcggattcacccttgtctgacctcaggcctctgaggggtgatgaactttttttttttctgagtgatc

SEQ ID NO: 11 - RNA, 78 nt, synthetic construct
  source 1..78: mol_type = other RNA
gatcacggtgatgagacccccccccctctgacctcaggcctctgaggggtgatgaacttgttgatggtctgagtgatc

SEQ ID NO: 12 - RNA, 78 nt, synthetic construct
  source 1..78: mol_type = other RNA
gatcacggtgatgagagctcggtacctctgacctcaggcctctgaggggtgatgaaccccccccccctctgagtgatc

SEQ ID NO: 13 - RNA, 78 nt, synthetic construct
  source 1..78: mol_type = other RNA
gatcacggtgatgagaactgatcgagtctgacctcaggcctctgaggggtgatgaacttgttgatggtctgagtgatc

SEQ ID NO: 14 - RNA, 78 nt, synthetic construct
  source 1..78: mol_type = other RNA
gatcacggtgatgagagctcggtacctctgacctcaggcctctgaggggtgatgaacactgatcgagtctgagtgatc

SEQ ID NO: 15 - RNA, 80 nt, synthetic construct
  source 1..80: mol_type = other RNA
ggatcacggtcctgagagctcggtacctctgacctcaggcctctgaggggtcctgaacttgttgatggtctgagtgatca

SEQ ID NO: 16 - RNA, 80 nt, synthetic construct
  source 1..80: mol_type = other RNA
ggatcacggtgatgagagctcggtacctctgacctcaggcctctgaggggtgatgaacttgttgatggtctccgtgatca

SEQ ID NO: 17 - RNA, 78 nt, synthetic construct
  source 1..78: mol_type = other RNA
gatcacggtgatgagagctcggtacctgtcgcctcaggcctctgaggggtgatgaacttgttgatggtgtcggtgatc

SEQ ID NO: 18 - RNA, 55 nt, synthetic construct
  source 1..55: mol_type = other RNA
gatcacggtgatgagatttttttttttctgacctcaggcctctgaggggtgatga

SEQ ID NO: 19 - RNA, 11 nt, synthetic construct
  source 1..11: mol_type = other RNA
tctgagtgatc

SEQ ID NO: 20 - RNA, 14 nt, synthetic construct
  source 1..14: mol_type = other RNA
gatcacggtgatga

SEQ ID NO: 21 - RNA, 52 nt, synthetic construct
  source 1..52: mol_type = other RNA
tctgacctcaggcctctgaggggtgatgagatttttttttttctgagtgatc

SEQ ID NO: 22 - RNA, 100 nt, synthetic construct
  source 1..100: mol_type = other RNA
gtcctttcctaataaaatgaggaaattgcatcgcattgggaaaaaaaaaaaaaaaaaaaaaaaaaaaaaaaaaaaaaaaaaaaaaaaaaaaaaaaaaaaa

SEQ ID NO: 23 - RNA, 100 nt, synthetic construct; identical to SEQ ID NO: 22
  source 1..100: mol_type = other RNA

SEQ ID NO: 24 - RNA, 100 nt, synthetic construct
  source 1..100: mol_type = other RNA
  modified_base 100: mod_base = OTHER; note = 2'-O-methyladenosine
gtcctttcctaataaaatgaggaaattgcatcgcattgggaaaaaaaaaaaaaaaaaaaaaaaaaaaaaaaaaaaaaaaaaaaaaaaaaaaaaaaaaaan

SEQ ID NO: 25 - RNA, 100 nt, synthetic construct
  source 1..100: mol_type = other RNA
  modified_base 70: mod_base = OTHER; note = 2'-O-methyladenosine
gtcctttcctaataaaatgaggaaattgcatcgcattgggaaaaaaaaaaaaaaaaaaaaaaaaaaaaanaaaaaaaaaaaaaaaaaaaaaaaaaaaaaa

SEQ ID NO: 26 - RNA, 100 nt, synthetic construct
  source 1..100: mol_type = other RNA
  modified_base 46: mod_base = OTHER; note = 2'-O-methyladenosine
gtcctttcctaataaaatgaggaaattgcatcgcattgggaaaaanaaaaaaaaaaaaaaaaaaaaaaaaaaaaaaaaaaaaaaaaaaaaaaaaaaaaaa

SEQ ID NO: 27 - RNA, 100 nt, synthetic construct
  source 1..100: mol_type = other RNA
  modified_base 56: mod_base = OTHER; note = 2'-O-methyladenosine
gtcctttcctaataaaatgaggaaattgcatcgcattgggaaaaaaaaaaaaaaanaaaaaaaaaaaaaaaaaaaaaaaaaaaaaaaaaaaaaaaaaaaa

SEQ ID NO: 28 - RNA, 100 nt, synthetic construct
  source 1..100: mol_type = other RNA
  modified_base 66: mod_base = OTHER; note = 2'-O-methyladenosine
gtcctttcctaataaaatgaggaaattgcatcgcattgggaaaaaaaaaaaaaaaaaaaaaaaaanaaaaaaaaaaaaaaaaaaaaaaaaaaaaaaaaaa

SEQ ID NO: 29 - RNA, 100 nt, synthetic construct
  source 1..100: mol_type = other RNA
  modified_base 76: mod_base = OTHER; note = 2'-O-methyladenosine
gtcctttcctaataaaatgaggaaattgcatcgcattgggaaaaaaaaaaaaaaaaaaaaaaaaaaaaaaaaaaanaaaaaaaaaaaaaaaaaaaaaaaa

SEQ ID NO: 30 - RNA, 100 nt, synthetic construct
  source 1..100: mol_type = other RNA
  modified_base 86: mod_base = OTHER; note = 2'-O-methyladenosine
gtcctttcctaataaaatgaggaaattgcatcgcattgggaaaaaaaaaaaaaaaaaaaaaaaaaaaaaaaaaaaaaaaaaaaaanaaaaaaaaaaaaaa

SEQ ID NO: 31 - RNA, 100 nt, synthetic construct
  source 1..100: mol_type = other RNA
  modified_base 96: mod_base = OTHER; note = 2'-O-methyladenosine
gtcctttcctaataaaatgaggaaattgcatcgcattgggaaaaaaaaaaaaaaaaaaaaaaaaaaaaaaaaaaaaaaaaaaaaaaaaaaaaaaanaaaa

SEQ ID NO: 32 - RNA, 20 nt, synthetic construct
  source 1..20: mol_type = other RNA
ggaaattgcatcgcattggg

SEQ ID NO: 33 - RNA, 20 nt, synthetic construct
  source 1..20: mol_type = other RNA
gtcctttcctaataaaatga

SEQ ID NO: 34 - RNA, 10 nt, synthetic construct
  source 1..10: mol_type = other RNA
ggttgggtca

SEQ ID NO: 35 - RNA, 10 nt, synthetic construct
  source 1..10: mol_type = other RNA
gtcccagcct

SEQ ID NO: 36 - RNA, 12 nt, synthetic construct
  source 1..12: mol_type = other RNA
gggggcggggcg

SEQ ID NO: 37 - RNA, 12 nt, synthetic construct
  source 1..12: mol_type = other RNA
gggctggcatat

SEQ ID NO: 38 - RNA, 12 nt, synthetic construct
  source 1..12: mol_type = other RNA
ggctgctcacca

SEQ ID NO: 39 - RNA, 12 nt, synthetic construct
  source 1..12: mol_type = other RNA
ggagctgagtcc

SEQ ID NO: 40 - RNA, 12 nt, synthetic construct
  source 1..12: mol_type = other RNA
ggggctggattt

SEQ ID NO: 41 - RNA, 12 nt, synthetic construct
  source 1..12: mol_type = other RNA
ggggttgggtca

SEQ ID NO: 42 - RNA, 12 nt, synthetic construct
  source 1..12: mol_type = other RNA
ggcccccttcct

SEQ ID NO: 43 - RNA, 12 nt, synthetic construct
  source 1..12: mol_type = other RNA
ggggggatcacg

SEQ ID NO: 44 - RNA, 12 nt, synthetic construct
  source 1..12: mol_type = other RNA
ggctttacagta

SEQ ID NO: 45 - RNA, 12 nt, synthetic construct
  source 1..12: mol_type = other RNA
ggggttggatcg

SEQ ID NO: 46 - RNA, 12 nt, synthetic construct
  source 1..12: mol_type = other RNA
ggaaagaggaac

SEQ ID NO: 47 - RNA, 12 nt, synthetic construct
  source 1..12: mol_type = other RNA
ggtgccctgcct

SEQ ID NO: 48 - RNA, 12 nt, synthetic construct
  source 1..12: mol_type = other RNA
ggattgctcact

SEQ ID NO: 49 - RNA, 12 nt, synthetic construct
  source 1..12: mol_type = other RNA
ggaggctttgca

SEQ ID NO: 50 - RNA, 10 nt, synthetic construct
  source 1..10: mol_type = other RNA
ggggatcacg

SEQ ID NO: 51 - RNA, 12 nt, synthetic construct
  source 1..12: mol_type = other RNA
ggattgtggcca

SEQ ID NO: 52 - RNA, 12 nt, synthetic construct
  source 1..12: mol_type = other RNA
ggcctatctctc

SEQ ID NO: 53 - RNA, 12 nt, synthetic construct
  source 1..12: mol_type = other RNA
ggatactttcct

SEQ ID NO: 54 - RNA, 15 nt, synthetic construct
  source 1..15: mol_type = other RNA
gctgccgccccatag

SEQ ID NO: 55 - RNA, 15 nt, synthetic construct
  source 1..15: mol_type = other RNA
tatgccagctcatag

SEQ ID NO: 56 - RNA, 15 nt, synthetic construct
  source 1..15: mol_type = other RNA
gctgtgagcccatag

SEQ ID NO: 57 - RNA, 15 nt, synthetic construct
  source 1..15: mol_type = other RNA
aactcagtttcatag

SEQ ID NO: 58 - RNA, 15 nt, synthetic construct
  source 1..15: mol_type = other RNA
agtccagcctcatag

SEQ ID NO: 59 - RNA, 15 nt, synthetic construct
  source 1..15: mol_type = other RNA
gtcccagcctcatag

SEQ ID NO: 60 - RNA, 15 nt, synthetic construct
  source 1..15: mol_type = other RNA
ggagatgggccatag

SEQ ID NO: 61 - RNA, 14 nt, synthetic construct
  source 1..14: mol_type = other RNA
gtgatcccccatag

SEQ ID NO: 62 - RNA, 15 nt, synthetic construct
  source 1..15: mol_type = other RNA
tgctgtttgccatag

SEQ ID NO: 63 - RNA, 15 nt, synthetic construct
  source 1..15: mol_type = other RNA
ggcccagcctcatag

SEQ ID NO: 64 - RNA, 15 nt, synthetic construct
  source 1..15: mol_type = other RNA
gtcctctgaccatag

SEQ ID NO: 65 - RNA, 15 nt, synthetic construct
  source 1..15: mol_type = other RNA
tggtggcacacatag

SEQ ID NO: 66 - RNA, 15 nt, synthetic construct
  source 1..15: mol_type = other RNA
gtgagcatctcatag

SEQ ID NO: 67 - RNA, 15 nt, synthetic construct
  source 1..15: mol_type = other RNA
gcaatgcctgcatag

SEQ ID NO: 68 - RNA, 12 nt, synthetic construct
  source 1..12: mol_type = other RNA
gtgatcacatag

SEQ ID NO: 69 - RNA, 15 nt, synthetic construct
  source 1..15: mol_type = other RNA
ggccaaattgcatag

SEQ ID NO: 70 - RNA, 15 nt, synthetic construct
  source 1..15: mol_type = other RNA
agaagagatgcatag

SEQ ID NO: 71 - RNA, 15 nt, synthetic construct
  source 1..15: mol_type = other RNA
ggaagggaggcatag

SEQ ID NO: 72 - RNA, 10 nt, synthetic construct
  source 1..10: mol_type = other RNA
ttttatgtgc

SEQ ID NO: 73 - RNA, 16 nt, synthetic construct
  source 1..16: mol_type = other RNA
gcaaagaaaggccttt

SEQ ID NO: 74 - RNA, 13 nt, synthetic construct
  source 1..13: mol_type = other RNA
aatgtttttcctt

SEQ ID NO: 75 - RNA, 10 nt, synthetic construct
  source 1..10: mol_type = other RNA
cagatcgact

SEQ ID NO: 76 - RNA, 13 nt, synthetic construct
  source 1..13: mol_type = other RNA
gattttttttttt

SEQ ID NO: 77 - RNA, 20 nt, synthetic construct
  source 1..20: mol_type = other RNA
agagtcacagtttgctgact

SEQ ID NO: 78 - RNA, 20 nt, synthetic construct
  source 1..20: mol_type = other RNA
atagtcacatataataaact

SEQ ID NO: 79 - RNA, 20 nt, synthetic construct
  source 1..20: mol_type = other RNA
gactccaaacatttgaatgt

SEQ ID NO: 80 - RNA, 20 nt, synthetic construct
  source 1..20: mol_type = other RNA
atggctaaacaaagtgcagt

SEQ ID NO: 81 - RNA, 20 nt, synthetic construct
  source 1..20: mol_type = other RNA
aactatctataaatggtact

SEQ ID NO: 82 - RNA, 20 nt, synthetic construct
  source 1..20: mol_type = other RNA
gaaaaagtactatggacagt

SEQ ID NO: 83 - RNA, 20 nt, synthetic construct
  source 1..20: mol_type = other RNA
ttcaattcagttagtgcagt

SEQ ID NO: 84 - RNA, 20 nt, synthetic construct
  source 1..20: mol_type = other RNA
taagtagttttaaggaaaat

SEQ ID NO: 85 - RNA, 87 nt, synthetic construct
  source 1..87: mol_type = other RNA
ggatcacggtgatgagatttttttttttctgacctcaggcctctgaggggtgatgaagagtcacagtttgctgactctgagtgatcc

SEQ ID NO: 86 - RNA, 87 nt, synthetic construct
  source 1..87: mol_type = other RNA
ggatcacggtgatgaagagtcacagtttgctgactctgacctcaggcctctgaggggtgatgagatttttttttttctgagtgatcc

SEQ ID NO: 87 - RNA, 87 nt, synthetic construct
  source 1..87: mol_type = other RNA
ggatcacggtgatgaatagtcacatataataaactctgacctcaggcctctgaggggtgatgagatttttttttttctgagtgatcc

SEQ ID NO: 88 - RNA, 87 nt, synthetic construct
  source 1..87: mol_type = other RNA
ggatcacggtgatgagatttttttttttctgacctcaggcctctgaggggtgatgaatagtcacatataataaactctgagtgatcc

SEQ ID NO: 89 - RNA, 87 nt, synthetic construct
  source 1..87: mol_type = other RNA
ggatcacggtgatgagatttttttttttctgacctcaggcctctgaggggtgatgagactccaaacatttgaatgtctgagtgatcc

SEQ ID NO: 90 - RNA, 87 nt, synthetic construct
  source 1..87: mol_type = other RNA
ggatcacggtgatgagactccaaacatttgaatgtctgacctcaggcctctgaggggtgatgagatttttttttttctgagtgatcc

SEQ ID NO: 91 - RNA, 87 nt, synthetic construct
  source 1..87: mol_type = other RNA
ggatcacggtgatgaatggctaaacaaagtgcagtctgacctcaggcctctgaggggtgatgagatttttttttttctgagtgatcc

SEQ ID NO: 92 - RNA, 87 nt, synthetic construct
  source 1..87: mol_type = other RNA
ggatcacggtgatgagatttttttttttctgacctcaggcctctgaggggtgatgaatggctaaacaaagtgcagtctgagtgatcc

SEQ ID NO: 93 - RNA, 87 nt, synthetic construct
  source 1..87: mol_type = other RNA
ggatcacggtgatgaaactatctataaatggtactctgacctcaggcctctgaggggtgatgagatttttttttttctgagtgatcc

SEQ ID NO: 94 - RNA, 87 nt, synthetic construct
  source 1..87: mol_type = other RNA
ggatcacggtgatgagatttttttttttctgacctcaggcctctgaggggtgatgaaactatctataaatggtactctgagtgatcc

SEQ ID NO: 95 - RNA, 87 nt, synthetic construct
  source 1..87: mol_type = other RNA
ggatcacggtgatgagaaaaagtactatggacagtctgacctcaggcctctgaggggtgatgagatttttttttttctgagtgatcc

SEQ ID NO: 96 - RNA, 87 nt, synthetic construct
  source 1..87: mol_type = other RNA
ggatcacggtgatgagatttttttttttctgacctcaggcctctgaggggtgatgagaaaaagtactatggacagtctgagtgatcc

SEQ ID NO: 97 - RNA, 87 nt, synthetic construct
  source 1..87: mol_type = other RNA
ggatcacggtgatgagatttttttttttctgacctcaggcctctgaggggtgatgattcaattcagttagtgcagtctgagtgatcc

SEQ ID NO: 98 - RNA, 87 nt, synthetic construct
  source 1..87: mol_type = other RNA
ggatcacggtgatgattcaattcagttagtgcagtctgacctcaggcctctgaggggtgatgagatttttttttttctgagtgatcc

SEQ ID NO: 99 - RNA, 87 nt, synthetic construct
  source 1..87: mol_type = other RNA
ggatcacggtgatgataagtagttttaaggaaaatctgacctcaggcctctgaggggtgatgagatttttttttttctgagtgatcc

SEQ ID NO: 100 - RNA, 87 nt, synthetic construct
  source 1..87: mol_type = other RNA
ggatcacggtgatgagatttttttttttctgacctcaggcctctgaggggtgatgataagtagttttaaggaaaatctgagtgatcc

SEQ ID NO: 101 - RNA, 85 nt, synthetic construct
  source 1..85: mol_type = other RNA
gatcacggtgatgagatttttttttttctgacctcaggcctctgaggggtgatgaagagtcacagtttgctgactctgagtgatc

SEQ ID NO: 102 - RNA, 85 nt, synthetic construct
  source 1..85: mol_type = other RNA
gatcacggtgatgaagagtcacagtttgctgactctgacctcaggcctctgaggggtgatgagatttttttttttctgagtgatc

SEQ ID NO: 103 - RNA, 85 nt, synthetic construct
  source 1..85: mol_type = other RNA
gatcacggtgatgaatagtcacatataataaactctgacctcaggcctctgaggggtgatgagatttttttttttctgagtgatc

SEQ ID NO: 104 - RNA, 85 nt, synthetic construct
  source 1..85: mol_type = other RNA
gatcacggtgatgagatttttttttttctgacctcaggcctctgaggggtgatgaatagtcacatataataaactctgagtgatc

SEQ ID NO: 105 - RNA, 85 nt, synthetic construct
  source 1..85: mol_type = other RNA
gatcacggtgatgagatttttttttttctgacctcaggcctctgaggggtgatgagactccaaacatttgaatgtctgagtgatc

SEQ ID NO: 106 - RNA, 85 nt, synthetic construct
  source 1..85: mol_type = other RNA
gatcacggtgatgagactccaaacatttgaatgtctgacctcaggcctctgaggggtgatgagatttttttttttctgagtgatc

SEQ ID NO: 107 - RNA, 85 nt, synthetic construct
  source 1..85: mol_type = other RNA
gatcacggtgatgaatggctaaacaaagtgcagtctgacctcaggcctctgaggggtgatgagatttttttttttctgagtgatc

SEQ ID NO: 108 - RNA, 85 nt, synthetic construct
  source 1..85: mol_type = other RNA
gatcacggtgatgagatttttttttttctgacctcaggcctctgaggggtgatgaatggctaaacaaagtgcagtctgagtgatc

SEQ ID NO: 109 - RNA, 85 nt, synthetic construct
  source 1..85: mol_type = other RNA
gatcacggtgatgaaactatctataaatggtactctgacctcaggcctctgaggggtgatgagatttttttttttctgagtgatc

SEQ ID NO: 110 - RNA, 85 nt, synthetic construct
  source 1..85: mol_type = other RNA
gatcacggtgatgagatttttttttttctgacctcaggcctctgaggggtgatgaaactatctataaatggtactctgagtgatc

SEQ ID NO: 111 - RNA, 86 nt, synthetic construct
  source 1..86: mol_type = other RNA
gatcacggtgatgagaaaaagtactatggacagtctgacctcaggcctctgaggggtgatgagatttttttttttctgagtgatcc

SEQ ID NO: 112 - RNA, 85 nt, synthetic construct
  source 1..85: mol_type = other RNA
gatcacggtgatgagatttttttttttctgacctcaggcctctgaggggtgatgagaaaaagtactatggacagtctgagtgatc

SEQ ID NO: 113 - RNA, 86 nt, synthetic construct
  source 1..86: mol_type = other RNA
ggatcacggtgatgagatttttttttttctgacctcaggcctctgaggggtgatgattcaattcagttagtgcagtctgagtgatc

SEQ ID NO: 114 - RNA, 85 nt, synthetic construct
  source 1..85: mol_type = other RNA
gatcacggtgatgattcaattcagttagtgcagtctgacctcaggcctctgaggggtgatgagatttttttttttctgagtgatc

SEQ ID NO: 115 - RNA, 85 nt, synthetic construct
  source 1..85: mol_type = other RNA
gatcacggtgatgataagtagttttaaggaaaatctgacctcaggcctctgaggggtgatgagatttttttttttctgagtgatc

SEQ ID NO: 116 - RNA, 85 nt, synthetic construct
  source 1..85: mol_type = other RNA
gatcacggtgatgagatttttttttttctgacctcaggcctctgaggggtgatgataagtagttttaaggaaaatctgagtgatc

SEQ ID NO: 117 - RNA, 81 nt, synthetic construct
  source 1..81: mol_type = other RNA
ggttgggtcaatgatgagatttttttttttctgaagagaggtgatgaagagtcacagtttgctgactctgagtcccagcct

SEQ ID NO: 118 - RNA, 81 nt, synthetic construct
  source 1..81: mol_type = other RNA
ggttgggtcaatgatgaagagtcacagtttgctgactctgaagagaggtgatgagatttttttttttctgagtcccagcct

SEQ ID NO: 119 - RNA, 81 nt, synthetic construct
  source 1..81: mol_type = other RNA
ggttgggtcaatgatgaatagtcacatataataaactctgaagagaggtgatgagatttttttttttctgagtcccagcct

SEQ ID NO: 120 - RNA, 81 nt, synthetic construct
  source 1..81: mol_type = other RNA
ggttgggtcaatgatgagatttttttttttctgaagagaggtgatgaatagtcacatataataaactctgagtcccagcct

SEQ ID NO: 121 - RNA, 81 nt, synthetic construct
  source 1..81: mol_type = other RNA
ggttgggtcaatgatgagatttttttttttctgaagagaggtgatgagactccaaacatttgaatgtctgagtcccagcct

SEQ ID NO: 122 - RNA, 81 nt, synthetic construct
  source 1..81: mol_type = other RNA
ggttgggtcaatgatgagactccaaacatttgaatgtctgaagagaggtgatgagatttttttttttctgagtcccagcct

SEQ ID NO: 123 - RNA, 81 nt, synthetic construct
  source 1..81: mol_type = other RNA
ggttgggtcaatgatgaatggctaaacaaagtgcagtctgaagagaggtgatgagatttttttttttctgagtcccagcct

SEQ ID NO: 124 - RNA, 81 nt, synthetic construct
  source 1..81: mol_type = other RNA
ggttgggtcaatgatgagatttttttttttctgaagagaggtgatgaatggctaaacaaagtgcagtctgagtcccagcct

SEQ ID NO: 125 - RNA, 81 nt, synthetic construct
  source 1..81: mol_type = other RNA
ggttgggtcaatgatgaaactatctataaatggtactctgaagagaggtgatgagatttttttttttctgagtcccagcct

SEQ ID NO: 126 - RNA, 81 nt, synthetic construct
  source 1..81: mol_type = other RNA
ggttgggtcaatgatgagatttttttttttctgaagagaggtgatgaaactatctataaatggtactctgagtcccagcct

SEQ ID NO: 127 - RNA, 81 nt, synthetic construct
  source 1..81: mol_type = other RNA
ggttgggtcaatgatgagaaaaagtactatggacagtctgaagagaggtgatgagatttttttttttctgagtcccagcct

SEQ ID NO: 128 - RNA, 81 nt, synthetic construct
  source 1..81: mol_type = other RNA
ggttgggtcaatgatgagatttttttttttctgaagagaggtgatgagaaaaagtactatggacagtctgagtcccagcct

SEQ ID NO: 129 - RNA, 81 nt, synthetic construct
  source 1..81: mol_type = other RNA
ggttgggtcaatgatgagatttttttttttctgaagagaggtgatgattcaattcagttagtgcagtctgagtcccagcct

SEQ ID NO: 130 - RNA, 81 nt, synthetic construct
  source 1..81: mol_type = other RNA
ggttgggtcaatgatgattcaattcagttagtgcagtctgaagagaggtgatgagatttttttttttctgagtcccagcct

SEQ ID NO: 131 - RNA, 81 nt, synthetic construct
  source 1..81: mol_type = other RNA
ggttgggtcaatgatgataagtagttttaaggaaaatctgaagagaggtgatgagatttttttttttctgagtcccagcct

SEQ ID NO: 132 - RNA, 81 nt, synthetic construct
  source 1..81: mol_type = other RNA
ggttgggtcaatgatgagatttttttttttctgaagagaggtgatgataagtagttttaaggaaaatctgagtcccagcct

SEQ ID NO: 133 - RNA, 88 nt, synthetic construct
  source 1..88: mol_type = other RNA
gggggcggggcggtgatgagatttttttttttctgagtgtcggtgctgaagagtcacagtttgctgactctgagctgccgccccatag

SEQ ID NO: 134 - RNA, 88 nt, synthetic construct
  source 1..88: mol_type = other RNA
gggggcggggcggtgatgaagagtcacagtttgctgactctgagtgtcggtgctgagatttttttttttctgagctgccgccccatag

SEQ ID NO: 135 - RNA, 88 nt, synthetic construct
  source 1..88: mol_type = other RNA
gggctggcatatatgatgagatttttttttttcagatcgactatgttgaagagtcacagtttgctgactctgatatgccagctcatag

SEQ ID NO: 136 - RNA, 88 nt, synthetic construct
  source 1..88: mol_type = other RNA
gggctggcatatatgatgaagagtcacagtttgctgactcagatcgactatgttgagatttttttttttctgatatgccagctcatag

SEQ ID NO: 137 - RNA, 93 nt, synthetic construct
  source 1..93: mol_type = other RNA
ggctgctcaccagtgatgagatttttttttttctgatcaatgtgtgactgaaagagagtcacagtttgctgactctgagctgtgagcccatag

SEQ ID NO: 138 - RNA, 93 nt, synthetic construct
  source 1..93: mol_type = other RNA
ggctgctcaccagtgatgaagagtcacagtttgctgactctgatcaatgtgtgactgaaaggatttttttttttctgagctgtgagcccatag

SEQ ID NO: 139 - RNA, 102 nt, synthetic construct
  source 1..102: mol_type = other RNA
ggagctgagtccatgatgagatttttttttttctgaaggcaaagaaaggcctttctgtgtggaagagtcacagtttgctgactctgaaactcagtttcatag

SEQ ID NO: 140 - RNA, 102 nt, synthetic construct
  source 1..102: mol_type = other RNA
ggagctgagtccatgatgaagagtcacagtttgctgactctgaaggcaaagaaaggcctttctgtgtggagatttttttttttctgaaactcagtttcatag

SEQ ID NO: 141 - RNA, 84 nt, synthetic construct
  source 1..84: mol_type = other RNA
ggggctggatttgtgatgagatttttttttttctgagcatgatgaagagtcacagtttgctgactctgaagtccagcctcatag

SEQ ID NO: 142 - RNA, 84 nt, synthetic construct
  source 1..84: mol_type = other RNA
ggggctggatttgtgatgaagagtcacagtttgctgactctgagcatgatgagatttttttttttctgaagtccagcctcatag

SEQ ID NO: 143 - RNA, 88 nt, synthetic construct
  source 1..88: mol_type = other RNA
ggggttgggtcaatgatgagatttttttttttctgaagagaggtgatgaagagtcacagtttgctgactctgagtcccagcctcatag

SEQ ID NO: 144 - RNA, 88 nt, synthetic construct
  source 1..88: mol_type = other RNA
ggggttgggtcaatgatgaagagtcacagtttgctgactctgaagagaggtgatgagatttttttttttctgagtcccagcctcatag

SEQ ID NO: 145 - RNA, 87 nt, synthetic construct
  source 1..87: mol_type = other RNA
ggcccccttcctatgatgagatttttttttttctgagctccgtgaggaagagtcacagtttgctgactctgaggagatgggccatag

SEQ ID NO: 146 - RNA, 87 nt, synthetic construct
  source 1..87: mol_type = other RNA
ggcccccttcctatgatgaagagtcacagtttgctgactctgagctccgtgaggagatttttttttttctgaggagatgggccatag

SEQ ID NO: 147 - RNA, 98 nt, synthetic construct
  source 1..98: mol_type = other RNA
ggggggatcacggtgatgagatttttttttttctgacctcaggcctctgaggggtgatgaagagtcacagtttgctgactctgagtgatcccccatag

SEQ ID NO: 148 - RNA, 98 nt, synthetic construct
  source 1..98: mol_type = other RNA
ggggggatcacggtgatgaagagtcacagtttgctgactctgacctcaggcctctgaggggtgatgagatttttttttttctgagtgatcccccatag

SEQ ID NO: 149 - RNA, 87 nt, synthetic construct
  source 1..87: mol_type = other RNA
ggctttacagtagtgatgagatttttttttttctgaaccacatgatttagagtcacagtttgctgactctgatgctgtttgccatag

SEQ ID NO: 150 - RNA, 87 nt, synthetic construct
  source 1..87: mol_type = other RNA
ggctttacagtagtgatgaagagtcacagtttgctgactctgaaccacatgatttgatttttttttttctgatgctgtttgccatag

SEQ ID NO: 151 - RNA, 88 nt, synthetic construct
  source 1..88: mol_type = other RNA
ggggttggatcgatgatgagatttttttttttctgaagagaggtgatgaagagtcacagtttgctgactctgaggcccagcctcatag

SEQ ID NO: 152 - RNA, 88 nt, synthetic construct
  source 1..88: mol_type = other RNA
ggggttggatcgatgatgaagagtcacagtttgctgactctgaagagaggtgatgagatttttttttttctgaggcccagcctcatag

SEQ ID NO: 153 - RNA, 88 nt, synthetic construct
  source 1..88: mol_type = other RNA
ggaaagaggaacatgaggagatttttttttttttgagtcaccaacatgtagagtcacagtttgctgactctgagtcctctgaccatag

SEQ ID NO: 154 - RNA, 88 nt, synthetic construct
  source 1..88: mol_type = other RNA
ggaaagaggaacatgaggaagagtcacagtttgctgactttgagtcaccaacatgtgatttttttttttctgagtcctctgaccatag

SEQ ID NO: 155 - RNA, 87 nt, synthetic construct
  source 1..87: mol_type = other RNA
ggtgccctgcctctgatgagatttttttttttctgagagtaatgatgaagagtcacagtttgctgactctgatggtggcacacatag

SEQ ID NO: 156 - RNA, 87 nt, synthetic construct
  source 1..87: mol_type = other RNA
ggtgccctgcctctgatgaagagtcacagtttgctgactctgagagtaatgatgagatttttttttttctgatggtggcacacatag

SEQ ID NO: 157 - RNA, 95 nt, synthetic construct
  source 1..95: mol_type = other RNA
ggattgctcactatgatgaagagtcacagtttgctgactcagaaatgtttttccttatgttgggatttttttttttctgagtgagcatctcatag

SEQ ID NO: 158 - RNA, 91 nt, synthetic construct
  source 1..91: mol_type = other RNA
ggaggctttgcagtgatgagatttttttttttctgagtgcaatcactgatgtagagtcacagtttgctgactctgagcaatgcctgcatag

SEQ ID NO: 159 - RNA, 91 nt, synthetic construct
  source 1..91: mol_type = other RNA
ggaggctttgcagtgatgaagagtcacagtttgctgactctgagtgcaatcactgatgtgatttttttttttctgagcaatgcctgcatag

SEQ ID NO: 160 - RNA, 94 nt, synthetic construct
  source 1..94: mol_type = other RNA
ggggatcacggtgatgagatttttttttttctgacctcaggcctctgaggggtgatgaagagtcacagtttgctgactctgagtgatcacatag

SEQ ID NO: 161 - RNA, 94 nt, synthetic construct
  source 1..94: mol_type = other RNA
ggggatcacggtgatgaagagtcacagtttgctgactctgacctcaggcctctgaggggtgatgagatttttttttttctgagtgatcacatag

SEQ ID NO: 162 - RNA, 99 nt, synthetic construct
  source 1..99: mol_type = other RNA
ggattgtggccaaggatgagatttttttttttctgattttatgtgcttctgctgtgatggagagtcacagtttgctgactctgaggccaaattgcatag

SEQ ID NO: 163 - RNA, 99 nt, synthetic construct
  source 1..99: mol_type = other RNA
ggattgtggccaaggatgaagagtcacagtttgctgactctgattttatgtgcttctgctgtgatgggatttttttttttctgaggccaaattgcatag

SEQ ID NO: 164 - RNA, 88 nt, synthetic construct
  source 1..88: mol_type = other RNA
ggcctatctctcatgatgaagagtcacagtttgctgactctgagctgctgtgatttgatttttttttttctgaagaagagatgcatag

SEQ ID NO: 165 - RNA, 88 nt, synthetic construct
  source 1..88: mol_type = other RNA
ggatactttcctctgatgaagagtcacagtttgctgactctgagacaccatgatgggatttttttttttctgaggaagggaggcatag

SEQ ID NO: 166 - RNA, 92 nt, synthetic construct
  source 1..92: mol_type = other RNA
gggctggcatatatgatgagatttttttttttccgacagatcgactatgttgaagagtcacagtttgctgactctgatatgccagctcatag

SEQ ID NO: 167 - RNA, 92 nt, synthetic construct
  source 1..92: mol_type = other RNA
gggctggcatatatgatgaagagtcacagtttgctgactccgacagatcgactatgttgagatttttttttttctgatatgccagctcatag

SEQ ID NO: 168 - RNA, 89 nt, synthetic construct
  source 1..89: mol_type = other RNA
ggctgctcaccagtgatgagatttttttttttctgatcaatgtgtgactgagagtcacagtttgctgactctgagctgtgagcccatag

SEQ ID NO: 169 - RNA, 89 nt, synthetic construct
  source 1..89: mol_type = other RNA
ggctgctcaccagtgatgaagagtcacagtttgctgactctgatcaatgtgtgactggatttttttttttctgagctgtgagcccatag

SEQ ID NO: 170 - RNA, 114 nt, synthetic construct
  source 1..114: mol_type = other RNA
  misc_difference 23..45: note = Each residue may individually be deleted so as to have a contiguous "n" sequence of between 7 to 30 contiguous "n" nucleotides
  misc_difference 81..103: note = Each residue may individually be deleted so as to have a contiguous "n" sequence of between 7 to 30 contiguous "n" nucleotides
ggatcacggtgatgannnnnnnnnnnnnnnnnnnnnnnnnnnnnnctgacctcaggcctctgaggggtgatgannnnnnnnnnnnnnnnnnnnnnnnnnnnnnctgagtgatcc

SEQ ID NO: 171 - RNA, 112 nt, synthetic construct
  source 1..112: mol_type = other RNA
  misc_difference 22..44: note = Each residue may individually be deleted so as to have a contiguous "n" sequence of between 7 to 30 contiguous "n" nucleotides
  misc_difference 80..102: note = Each residue may individually be deleted so as to have a contiguous "n" sequence of between 7 to 30 contiguous "n" nucleotides
gatcacggtgatgannnnnnnnnnnnnnnnnnnnnnnnnnnnnnctgacctcaggcctctgaggggtgatgannnnnnnnnnnnnnnnnnnnnnnnnnnnnnctgagtgatc

SEQ ID NO: 172 - RNA, 108 nt, synthetic construct
  source 1..108: mol_type = other RNA
  misc_difference 25..47: note = Each residue may individually be deleted so as to have a contiguous "n" sequence of between 7 to 30 contiguous "n" nucleotides
  misc_difference 72..94: note = Each residue may individually be deleted so as to have a contiguous "n" sequence of between 7 to 30 contiguous "n" nucleotides
ggttgggtcaatgatgannnnnnnnnnnnnnnnnnnnnnnnnnnnnnctgaagagaggtgatgannnnnnnnnnnnnnnnnnnnnnnnnnnnnnctgagtcccagcct

SEQ ID NO: 173 - RNA, 115 nt, synthetic construct
  source 1..115: mol_type = other RNA
  misc_difference 27..49: note = Each residue within the Feature Location may individually be deleted
  misc_difference 74..96: note = Each residue within the Feature Location may individually be deleted
gggggcggggcggtgatgannnnnnnnnnnnnnnnnnnnnnnnnnnnnnctgagtgtcggtgctgannnnnnnnnnnnnnnnnnnnnnnnnnnnnnctgagctgccgccccatag

SEQ ID NO: 174 - RNA, 115 nt, synthetic construct
  source 1..115: mol_type = other RNA
  misc_difference 27..49: note = Each residue within the Feature Location may individually be deleted
  misc_difference 74..96: note = Each residue within the Feature Location may individually be deleted
gggctggcatatatgatgannnnnnnnnnnnnnnnnnnnnnnnnnnnnncagatcgactatgttgannnnnnnnnnnnnnnnnnnnnnnnnnnnnnctgatatgccagctcatag

SEQ ID NO: 175 - RNA, 120 nt, synthetic construct
  source 1..120: mol_type = other RNA
  misc_difference 27..49: note = Each residue within the Feature Location may individually be deleted
  misc_difference 79..101: note = Each residue within the Feature Location may individually be deleted
ggctgctcaccagtgatgannnnnnnnnnnnnnnnnnnnnnnnnnnnnnctgatcaatgtgtgactgaaagnnnnnnnnnnnnnnnnnnnnnnnnnnnnnnctgagctgtgagcccatag

SEQ ID NO: 176 - RNA, 129 nt, synthetic construct
  source 1..129: mol_type = other RNA
  misc_difference 27..49: note = Each residue within the Feature Location may individually be deleted
  misc_difference 88..110: note = Each residue within the Feature Location may individually be deleted
ggagctgagtccatgatgannnnnnnnnnnnnnnnnnnnnnnnnnnnnnctgaaggcaaagaaaggcctttctgtgtggannnnnnnnnnnnnnnnnnnnnnnnnnnnnnctgaaactcagtttcatag

SEQ ID NO: 177 - RNA, 111 nt, synthetic construct
  source 1..111: mol_type = other RNA
  misc_difference 27..49: note = Each residue within the Feature Location may individually be deleted
  misc_difference 70..92: note = Each residue within the Feature Location may individually be deleted
ggggctggatttgtgatgannnnnnnnnnnnnnnnnnnnnnnnnnnnnnctgagcatgatgannnnnnnnnnnnnnnnnnnnnnnnnnnnnnctgaagtccagcctcatag

SEQ ID NO: 178 - RNA, 115 nt, synthetic construct
  source 1..115: mol_type = other RNA
  misc_difference 27..49: note = Each residue within the Feature Location may individually be deleted
  misc_difference 74..96: note = Each residue within the Feature Location may individually be deleted
ggggttgggtcaatgatgannnnnnnnnnnnnnnnnnnnnnnnnnnnnnctgaagagaggtgatgannnnnnnnnnnnnnnnnnnnnnnnnnnnnnctgagtcccagcctcatag

SEQ ID NO: 179 - RNA, 114 nt, synthetic construct
  source 1..114: mol_type = other RNA
  misc_difference 27..49: note = Each residue within the Feature Location may individually be deleted
  misc_difference 73..95: note = Each residue within the Feature Location may individually be deleted
ggcccccttcctatgatgannnnnnnnnnnnnnnnnnnnnnnnnnnnnnctgagctccgtgaggannnnnnnnnnnnnnnnnnnnnnnnnnnnnnctgaggagatgggccatag

SEQ ID NO: 180 - RNA, 125 nt, synthetic construct
  source 1..125: mol_type = other RNA
  misc_difference 27..49: note = Each residue within the Feature Location may individually be deleted
  misc_difference 85..107: note = Each residue within the Feature Location may individually be deleted
ggggggatcacggtgatgannnnnnnnnnnnnnnnnnnnnnnnnnnnnnctgacctcaggcctctgaggggtgatgannnnnnnnnnnnnnnnnnnnnnnnnnnnnnctgagtgatcccccatag

SEQ ID NO: 181 - RNA, 114 nt, synthetic construct
  source 1..114: mol_type = other RNA
  misc_difference 27..49: note = Each residue within the Feature Location may individually be deleted
  misc_difference 73..95: note = Each residue within the Feature Location may individually be deleted
ggctttacagtagtgatgannnnnnnnnnnnnnnnnnnnnnnnnnnnnnctgaaccacatgatttnnnnnnnnnnnnnnnnnnnnnnnnnnnnnnctgatgctgtttgccatag

SEQ ID NO: 182 - RNA, 115 nt, synthetic construct
  source 1..115: mol_type = other RNA
  misc_difference 27..49: note = Each residue within the Feature Location may individually be deleted
  misc_difference 74..96: note = Each residue within the Feature Location may individually be deleted
ggggttggatcgatgatgannnnnnnnnnnnnnnnnnnnnnnnnnnnnnctgaagagaggtgatgannnnnnnnnnnnnnnnnnnnnnnnnnnnnnctgaggcccagcctcatag

SEQ ID NO: 183 - RNA, 115 nt, synthetic construct
  source 1..115: mol_type = other RNA
  misc_difference 27..49: note = Each residue within the Feature Location may individually be deleted
  misc_difference 74..96: note = Each residue within the Feature Location may individually be deleted
ggaaagaggaacatgaggannnnnnnnnnnnnnnnnnnnnnnnnnnnnnttgagtcaccaacatgtnnnnnnnnnnnnnnnnnnnnnnnnnnnnnnctgagtcctctgaccatag

SEQ ID NO: 184 - RNA, 114 nt, synthetic construct
  source 1..114: mol_type = other RNA
  misc_difference 27..49: note = Each residue within the Feature Location may individually be deleted
  misc_difference 73..95: note = Each residue within the Feature Location may individually be deleted
ggtgccctgcctctgatgannnnnnnnnnnnnnnnnnnnnnnnnnnnnnctgagagtaatgatgannnnnnnnnnnnnnnnnnnnnnnnnnnnnnctgatggtggcacacatag

SEQ ID NO: 185 - RNA, 122 nt, synthetic construct
  source 1..122: mol_type = other RNA
  misc_difference 27..49: note = Each residue within the Feature Location may individually be deleted
  misc_difference 81..103: note = Each residue within the Feature Location may individually be deleted
ggattgctcactatgatgannnnnnnnnnnnnnnnnnnnnnnnnnnnnncagaaatgtttttccttatgttggnnnnnnnnnnnnnnnnnnnnnnnnnnnnnnctgagtgagcatctcatag

SEQ ID NO: 186 - RNA, 118 nt, synthetic construct
  source 1..118: mol_type = other RNA
  misc_difference 27..49: note = Each residue within the Feature Location may individually be deleted
  misc_difference 77..99: note = Each residue within the Feature Location may individually be deleted
ggaggctttgcagtgatgannnnnnnnnnnnnnnnnnnnnnnnnnnnnnctgagtgcaatcactgatgtnnnnnnnnnnnnnnnnnnnnnnnnnnnnnnctgagcaatgcctgcatag

SEQ ID NO: 187 - RNA, 121 nt, synthetic construct
  source 1..121: mol_type = other RNA
  misc_difference 25..47: note = Each residue within the Feature Location may individually be deleted
  misc_difference 83..105: note = Each residue within the Feature Location may individually be deleted
ggggatcacggtgatgannnnnnnnnnnnnnnnnnnnnnnnnnnnnnctgacctcaggcctctgaggggtgatgannnnnnnnnnnnnnnnnnnnnnnnnnnnnnctgagtgatcacatag

SEQ ID NO: 188 - RNA, 126 nt, synthetic construct
  source 1..126: mol_type = other RNA
  misc_difference 27..49: note = Each residue within the Feature Location may individually be deleted
  misc_difference 85..107: note = Each residue within the Feature Location may individually be deleted
ggattgtggccaaggatgannnnnnnnnnnnnnnnnnnnnnnnnnnnnnctgattttatgtgcttctgctgtgatggnnnnnnnnnnnnnnnnnnnnnnnnnnnnnnctgaggccaaattgcatag

SEQ ID NO: 189 - RNA, 115 nt, synthetic construct
  source 1..115: mol_type = other RNA
  misc_difference 27..49: note = Each residue within the Feature Location may individually be deleted
  misc_difference 74..96: note = Each residue within the Feature Location may individually be deleted
ggcctatctctcatgatgannnnnnnnnnnnnnnnnnnnnnnnnnnnnnctgagctgctgtgatttnnnnnnnnnnnnnnnnnnnnnnnnnnnnnnctgaagaagagatgcatag

SEQ ID NO: 190 - RNA, 115 nt, synthetic construct
  source 1..115: mol_type = other RNA
  misc_difference 27..49: note = Each residue within the Feature Location may individually be deleted
  misc_difference 74..96: note = Each residue within the Feature Location may individually be deleted
ggatactttcctctgatgannnnnnnnnnnnnnnnnnnnnnnnnnnnnnctgagacaccatgatggnnnnnnnnnnnnnnnnnnnnnnnnnnnnnnctgaggaagggaggcatag

SEQ ID NO: 191 - RNA, 119 nt, synthetic construct
  source 1..119: mol_type = other RNA
  misc_difference 27..49: note = Each residue within the Feature Location may individually be deleted
  misc_difference 78..100: note = Each residue within the Feature Location may individually be deleted
gggctggcatatatgatgannnnnnnnnnnnnnnnnnnnnnnnnnnnnnccgacagatcgactatgttgannnnnnnnnnnnnnnnnnnnnnnnnnnnnnctgatatgccagctcatag

SEQ ID NO: 192 - RNA, 116 nt, synthetic construct
  source 1..116: mol_type = other RNA
  misc_difference 27..49: note = Each residue within the Feature Location may individually be deleted
  misc_difference 75..97: note = Each residue within the Feature Location may individually be deleted
ggctgctcaccagtgatgannnnnnnnnnnnnnnnnnnnnnnnnnnnnnctgatcaatgtgtgactgnnnnnnnnnnnnnnnnnnnnnnnnnnnnnnctgagctgtgagcccatag